European Patent Application EP 4 600 356 A1, published August 13, 2025. Title: Method for introducing a nucleic acid to mitochondria. Applicant: RIKEN. Application JP. The sequence listing filed with the application follows.

SEQUENCE LISTING (43 sequences)

SEQ ID NO: 1 - protein, 19 aa, Homo sapiens
IAAVTIAAGTAAIGYLAYK

SEQ ID NO: 2 - protein, 32 aa, Homo sapiens
MSLTSSSSVRVEWIAAVTIAAGTAAIGYLAYK

SEQ ID NO: 3 - protein, 18 aa, synthetic construct
RHRHRHRHRHRHRHRHRH

SEQ ID NO: 4 - protein, 18 aa, synthetic construct
KHKHKHKHKHKHKHKHKH

SEQ ID NO: 5 - protein, 50 aa, synthetic construct
MSLTSSSSVRVEWIAAVTIAAGTAAIGYLAYKRHRHRHRHRHRHRHRHRH

SEQ ID NO: 6 - protein, 50 aa, synthetic construct
MSLTSSSSVRVEWIAAVTIAAGTAAIGYLAYKKHKHKHKHKHKHKHKHKH

SEQ ID NO: 7 - protein, 9 aa, synthetic construct
RKKRRQRRR

SEQ ID NO: 8 - protein, 27 aa, synthetic construct
RKKRRQRRRRHRHRHRHRHRHRHRHRH

SEQ ID NO: 9 - DNA, 20 bp, synthetic construct
  source 1..20: mol_type = other DNA
ccctaaaacccgccacatct

SEQ ID NO: 10 - DNA, 22 bp, synthetic construct
  source 1..22: mol_type = other DNA
agcgatggtgagagctaaggtc

SEQ ID NO: 11 - DNA, 21 bp, synthetic construct
  source 1..21: mol_type = other DNA
gccttctccacttcaagtcaa

SEQ ID NO: 12 - DNA, 21 bp, synthetic construct
  source 1..21: mol_type = other DNA
tgggtacagatgtgcaggaat

SEQ ID NO: 13 - DNA, 20 bp, synthetic construct
  source 1..20: mol_type = other DNA
atcgtgcgggacatcaagga

SEQ ID NO: 14 - DNA, 20 bp, synthetic construct
  source 1..20: mol_type = other DNA
aggaaggagggctggaagag

SEQ ID NO: 15 - protein, 12 aa, Saccharomyces cerevisiae
MLSLRQSIRFFK

SEQ ID NO: 16 - protein, 30 aa, synthetic construct
MLSLRQSIRFFKKHKHKHKHKHKHKHKHKH

SEQ ID NO: 17 - protein, 108 aa, Homo sapiens
MSLTSSSSVRVEWIAAVTIAAGTAAIGYLAYKRFYVKDHRNKAMINLHIQKDNPKIVHAFDMEDLGDKAVYCRCWRSKKFPFCDGAHTKHNEETGDNVGPLIIKKKET

SEQ ID NO: 18 - DNA, 327 bp, Homo sapiens
  source 1..327: mol_type = other DNA
atgagtctgacttccagttccagcgtacgagttgaatggatcgcagcagttaccattgctgctgggacagctgcaattggttatctagcttacaaaagattttatgttaaagatcatcgaaataaagctatgataaaccttcacatccagaaagacaaccccaagatagtacatgcttttgacatggaggatttgggagataaagctgtgtactgccgttgttggaggtccaaaaagttcccattctgtgatggggctcacacaaaacataacgaagagactggagacaatgtgggccctctgatcatcaagaaaaaagaaacttaa

SEQ ID NO: 19 - protein, 8 aa, synthetic construct
KKKKKKKK

SEQ ID NO: 20 - protein, 108 aa, Mus musculus
MGLSSNSAVRVEWIAAVTFAAGTAALGYLAYKKFYAKENRTKAMVNLQIQKDNPKVVHAFDMEDLGDKAVYCRCWRSKKFPFCDGAHIKHNEETGDNVGPLIIKKKET

SEQ ID NO: 21 - protein, 19 aa, Mus musculus
IAAVTFAAGTAALGYLAYK

SEQ ID NO: 22 - protein, 32 aa, Mus musculus
MGLSSNSAVRVEWIAAVTFAAGTAALGYLAYK

SEQ ID NO: 23 - protein, 106 aa, Bos taurus
MSMTSSVRVEWIAAVTIAAGTAAIGYLAYKRFYVKDHRNKSMVNPHIQKDNPKVVHAFDMEDLGDKAVYCRCWRSKKFPLCDGSHTKHNEETGDNVGPLIIKKKDT

SEQ ID NO: 24 - protein, 19 aa, Bos taurus
IAAVTIAAGTAAIGYLAYK

SEQ ID NO: 25 - protein, 30 aa, Bos taurus
MSMTSSVRVEWIAAVTIAAGTAAIGYLAYK

SEQ ID NO: 26 - protein, 101 aa, Anas platyrhynchos
SVSEWLRLLPFLGVLALLGYLAVRPFLHKKKQQKDSLINLKIQKENPKVVNEINIEDLCLTKAYCRCWRSKTFPVCDGSHNKHNELTGDNVGPLILKKKEV

SEQ ID NO: 27 - protein, 19 aa, Anas platyrhynchos
LRLLPFLGVLALLGYLAVR

SEQ ID NO: 28 - protein, 24 aa, Anas platyrhynchos
SVSEWLRLLPFLGVLALLGYLAVR

SEQ ID NO: 29 - protein, 135 aa, Salmo salar
MVLETISRIIKIQLPAYLKKLPLPETIGGFARLTVSEWLRLLPLLGILALLGYLTIRPFLPKKKKQKDSLINLKIQKENPKVVNEIDIEDLKRTNVCYCRCWRSKTFPVCDKSHIKHNELTGDNVGPLILKKKIL

SEQ ID NO: 30 - protein, 19 aa, Salmo salar
LRLLPLLGILALLGYLTIR

SEQ ID NO: 31 - protein, 57 aa, Salmo salar
MVLETISRIIKIQLPAYLKKLPLPETIGGFARLTVSEWLRLLPLLGILALLGYLTIR

SEQ ID NO: 32 - protein, 134 aa, Drosophila melanogaster
MESLSQLVKSTLPNYLSNLPIPDSVGGWFKLSFKDWLALIPPTVVVAGIGYTGYLAFCPAAQARCSATKSGRCNNQIRKHEPKVVDTIDVEDIADKAAFCRCWKSKNWPYCDGSHGEHNKLTGDNVGPVVVKKQ

SEQ ID NO: 33 - protein, 19 aa, Drosophila melanogaster
LALIPPTVVVAGIGYTGYL

SEQ ID NO: 34 - protein, 55 aa, Drosophila melanogaster
MESLSQLVKSTLPNYLSNLPIPDSVGGWFKLSFKDWLALIPPTVVVAGIGYTGYL

SEQ ID NO: 35 - protein, 107 aa, Danio rerio
MSASNSFHKAEIIAAVSVTFGAAAVGLLVYKTFFHNSKCVKPKVNLDLQKDNPKVVHAFDIEDLGDKAVYCRCWRSKKFPFCDGAHAKHNQETGDNVGPLIIKRKEA

SEQ ID NO: 36 - protein, 19 aa, Danio rerio
IAAVSVTFGAAAVGLLVYK

SEQ ID NO: 37 - protein, 31 aa, Danio rerio
MSASNSFHKAEIIAAVSVTFGAAAVGLLVYK

SEQ ID NO: 38 - protein, 103 aa, Caenorhabditis elegans
MPCPTQVSGRCVATTAAVLAGGALIGYLVGYKFGQRSARCNYKIQLDSNKIVDTVDIEDIGEKKAFCRCWKSEKWPYCDGSHGKHNKETGDNVGPLIVKSEKK

SEQ ID NO: 39 - protein, 17 aa, Caenorhabditis elegans
TTAAVLAGGALIGYLVG

SEQ ID NO: 40 - protein, 30 aa, Caenorhabditis elegans
MPCPTQVSGRCVATTAAVLAGGALIGYLVG

SEQ ID NO: 41 - protein, 108 aa, Arabidopsis thaliana
MAIIASTFGTGLSYAGELPFKPVTGGEVGRKQQRMVVVRAEGGGGINPEIRKNEDKVVDSVVVTELSKNITPYCRCWRSGTFPLCDGSHVKHNKANGDNVGPLLLKKQ

SEQ ID NO: 42 - protein, 18 aa, Arabidopsis thaliana
AGELPFKPVTGGEVGRKQ

SEQ ID NO: 43 - protein, 32 aa, Arabidopsis thaliana
MAIIASTFGTGLSYAGELPFKPVTGGEVGRKQ